European Patent Application EP 4 194 468 A1, published June 14, 2023. Title: ANTI-PD-L1 ANTIBODY AND USE THEREOF. Applicant: Bio-Thera Solutions, Ltd. Application EP 21 853 735.5. The sequence listing filed with the application follows.

SEQUENCE LISTING (107 sequences)

SEQ ID NO: 1 - protein, 10 aa, Artificial Sequence
GFTFSDSWIH

SEQ ID NO: 2 - protein, 10 aa, Artificial Sequence
SFSLKDSWIH

SEQ ID NO: 3 - protein, 10 aa, Artificial Sequence
GWATRDSWIH

SEQ ID NO: 4 - protein, 10 aa, Artificial Sequence
NSHLRDSWIH

SEQ ID NO: 5 - protein, 10 aa, Artificial Sequence
GLRPADSWIH

SEQ ID NO: 6 - protein, 10 aa, Artificial Sequence
GFTFSDSWIH

SEQ ID NO: 7 - protein, 18 aa, Artificial Sequence
GWISPYGGSTYYADDFRH

SEQ ID NO: 8 - protein, 18 aa, Artificial Sequence
GWISPYGGSTYYADSLGD

SEQ ID NO: 9 - protein, 18 aa, Artificial Sequence
GWISPYGGSTYYADHLSQ

SEQ ID NO: 10 - protein, 18 aa, Artificial Sequence
GWISPYGGSTYYADGMRS

SEQ ID NO: 11 - protein, 18 aa, Artificial Sequence
GWISPYGGSTYYADSYRS

SEQ ID NO: 12 - protein, 18 aa, Artificial Sequence
GWISPYGGSTYYADPYVG

SEQ ID NO: 13 - protein, 18 aa, Artificial Sequence
GWISPYGGSTYYADSLKG

SEQ ID NO: 14 - protein, 18 aa, Artificial Sequence
GWISPYGGSTYYADSYRA

SEQ ID NO: 15 - protein, 18 aa, Artificial Sequence
GWISPYGGSTYYADYLHG

SEQ ID NO: 16 - protein, 18 aa, Artificial Sequence
GWISPYGGSTYYADSVKG

SEQ ID NO: 17 - protein, 9 aa, Artificial Sequence
RHWPGGFDY

SEQ ID NO: 18 - protein, 9 aa, Artificial Sequence
RHWPGGLLP

SEQ ID NO: 19 - protein, 11 aa, Artificial Sequence
LASQTIGTWLA

SEQ ID NO: 20 - protein, 11 aa, Artificial Sequence
QASQDIGKHLN

SEQ ID NO: 21 - protein, 11 aa, Artificial Sequence
RASQGIGSWLA

SEQ ID NO: 22 - protein, 11 aa, Artificial Sequence
RASQGISSYLA

SEQ ID NO: 23 - protein, 11 aa, Artificial Sequence
RASQGIGKFLA

SEQ ID NO: 24 - protein, 7 aa, Artificial Sequence
AASTLQS

SEQ ID NO: 25 - protein, 7 aa, Artificial Sequence
GASNLKT

SEQ ID NO: 26 - protein, 7 aa, Artificial Sequence
AASSLQS

SEQ ID NO: 27 - protein, 7 aa, Artificial Sequence
AASRLQS

SEQ ID NO: 28 - protein, 9 aa, Artificial Sequence
QQYYSTPRT

SEQ ID NO: 29 - protein, 9 aa, Artificial Sequence
QQSYTTPYT

SEQ ID NO: 30 - protein, 9 aa, Artificial Sequence
QQYFSTPYT

SEQ ID NO: 31 - protein, 9 aa, Artificial Sequence
QQYYSTPYT

SEQ ID NO: 32 - protein, 25 aa, Artificial Sequence [sequence omitted]

SEQ ID NO: 33 - protein, 13 aa, Artificial Sequence
WVRQAPGKGLEWV

SEQ ID NO: 34 - protein, 32 aa, Artificial Sequence
RFTISADTSKNTAYLQMNSLRAEDTAVYYCAR

SEQ ID NO: 35 - protein, 11 aa, Artificial Sequence
WGQGTLVTVSS

SEQ ID NO: 36 - protein, 118 aa, Artificial Sequence
EVQLVESGGGLVQPGGSLRLSCAASGFTFSDSWIHWVRQAPGKGLEWVGWISPYGGSTYYADSVKGRFTISADTSKNTAYLQMNSLRAEDTAVYYCARRHWPGGFDYWGQGTLVTVSS

SEQ ID NO: 37 - protein, 118 aa, Artificial Sequence
EVQLVESGGGLVQPGGSLRLSCAASGFTFSDSWIHWVRQAPGKGLEWVGWISPYGGSTYYADDFRHRFTISADTSKNTAYLQMNSLRAEDTAVYYCARRHWPGGFDYWGQGTLVTVSS

SEQ ID NO: 38 - protein, 118 aa, Artificial Sequence
EVQLVESGGGLVQPGGSLRLSCAASGFTFSDSWIHWVRQAPGKGLEWVGWISPYGGSTYYADSLGDRFTISADTSKNTAYLQMNSLRAEDTAVYYCARRHWPGGFDYWGQGTLVTVSS

SEQ ID NO: 39 - protein, 118 aa, Artificial Sequence
EVQLVESGGGLVQPGGSLRLSCAASGFTFSDSWIHWVRQAPGKGLEWVGWISPYGGSTYYADHLSQRFTISADTSKNTAYLQMNSLRAEDTAVYYCARRHWPGGFDYWGQGTLVTVSS

SEQ ID NO: 40 - protein, 118 aa, Artificial Sequence
EVQLVESGGGLVQPGGSLRLSCAASGFTFSDSWIHWVRQAPGKGLEWVGWISPYGGSTYYADGMRSRFTISADTSKNTAYLQMNSLRAEDTAVYYCARRHWPGGFDYWGQGTLVTVSS

SEQ ID NO: 41 - protein, 118 aa, Artificial Sequence
EVQLVESGGGLVQPGGSLRLSCAASGFTFSDSWIHWVRQAPGKGLEWVGWISPYGGSTYYADSYRSRFTISADTSKNTAYLQMNSLRAEDTAVYYCARRHWPGGFDYWGQGTLVTVSS

SEQ ID NO: 42 - protein, 118 aa, Artificial Sequence
EVQLVESGGGLVQPGGSLRLSCAASGFTFSDSWIHWVRQAPGKGLEWVGWISPYGGSTYYADPYVGRFTISADTSKNTAYLQMNSLRAEDTAVYYCARRHWPGGFDYWGQGTLVTVSS

SEQ ID NO: 43 - protein, 118 aa, Artificial Sequence
EVQLVESGGGLVQPGGSLRLSCAASGFTFSDSWIHWVRQAPGKGLEWVGWISPYGGSTYYADSLKGRFTISADTSKNTAYLQMNSLRAEDTAVYYCARRHWPGGFDYWGQGTLVTVSS

SEQ ID NO: 44 - protein, 118 aa, Artificial Sequence
EVQLVESGGGLVQPGGSLRLSCAASGFTFSDSWIHWVRQAPGKGLEWVGWISPYGGSTYYADSYRARFTISADTSKNTAYLQMNSLRAEDTAVYYCARRHWPGGFDYWGQGTLVTVSS

SEQ ID NO: 45 - protein, 118 aa, Artificial Sequence
EVQLVESGGGLVQPGGSLRLSCAASGFTFSDSWIHWVRQAPGKGLEWVGWISPYGGSTYYADYLHGRFTISADTSKNTAYLQMNSLRAEDTAVYYCARRHWPGGFDYWGQGTLVTVSS

SEQ ID NO: 46 - protein, 118 aa, Artificial Sequence
EVQLVESGGGLVQPGGSLRLSCAASSFSLKDSWIHWVRQAPGKGLEWVGWISPYGGSTYYADSVKGRFTISADTSKNTAYLQMNSLRAEDTAVYYCARRHWPGGFDYWGQGTLVTVSS

SEQ ID NO: 47 - protein, 118 aa, Artificial Sequence
EVQLVESGGGLVQPGGSLRLSCAASGWATRDSWIHWVRQAPGKGLEWVGWISPYGGSTYYADSVKGRFTISADTSKNTAYLQMNSLRAEDTAVYYCARRHWPGGFDYWGQGTLVTVSS

SEQ ID NO: 48 - protein, 118 aa, Artificial Sequence
EVQLVESGGGLVQPGGSLRLSCAASGFTFSDSWIHWVRQAPGKGLEWVGWISPYGGSTYYADSVKGRFTISADTSKNTAYLQMNSLRAEDTAVYYCARRHWPGGLLPWGQGTLVTVSS

SEQ ID NO: 49 - protein, 118 aa, Artificial Sequence
EVQLVESGGGLVQPGGSLRLSCAASGLRPADSWIHWVRQAPGKGLEWVGWISPYGGSTYYADSVKGRFTISADTSKNTAYLQMNSLRAEDTAVYYCARRHWPGGFDYWGQGTLVTVSS

SEQ ID NO: 50 - protein, 118 aa, Artificial Sequence
EVQLVESGGGLVQPGGSLRLSCAASNSHLRDSWIHWVRQAPGKGLEWVGWISPYGGSTYYADSVKGRFTISADTSKNTAYLQMNSLRAEDTAVYYCARRHWPGGFDYWGQGTLVTVSS

SEQ ID NO: 51 - protein, 23 aa, Artificial Sequence
EIVLTQSPSSLSASVGDRVTITC

SEQ ID NO: 52 - protein, 23 aa, Artificial Sequence
EIVLTQSPSSVSASVGDKLTMTC

SEQ ID NO: 53 - protein, 23 aa, Artificial Sequence
EIVLTQSPSSVSASVGDRITITC

SEQ ID NO: 54 - protein, 23 aa, Artificial Sequence
DIQMTQSPSSFSASTGDRVTITC

SEQ ID NO: 55 - protein, 23 aa, Artificial Sequence
DIQMTQSPSSLSASVGDRVTIPC

SEQ ID NO: 56 - protein, 23 aa, Artificial Sequence
DIQMTQSPSSLSASVGDRVTITC

SEQ ID NO: 57 - protein, 15 aa, Artificial Sequence
WYQQKPGKSPQLLIY

SEQ ID NO: 58 - protein, 15 aa, Artificial Sequence
WYQQKPGKPPKLLIY

SEQ ID NO: 59 - protein, 15 aa, Artificial Sequence
WYQQKPGKAPSLLIY

SEQ ID NO: 60 - protein, 15 aa, Artificial Sequence
WYQQKPGKAPKLLIY

SEQ ID NO: 61 - protein, 32 aa, Artificial Sequence
GVPSRFSGSGSGTDFTLTISSLQPEDVATYYC

SEQ ID NO: 62 - protein, 32 aa, Artificial Sequence
GVPSRFSGTGSGTDFTLTISSLQPEDFATYYC

SEQ ID NO: 63 - protein, 32 aa, Artificial Sequence
GVPSRFSGSGSGTDFTLTISSLQTEDVAVYYC

SEQ ID NO: 64 - protein, 32 aa, Artificial Sequence
GVPSRFSGSGSGTDFTLTISSLQAEDVAVYYC

SEQ ID NO: 65 - protein, 10 aa, Artificial Sequence
FGQGTKVEIK

SEQ ID NO: 66 - protein, 10 aa, Artificial Sequence
FGQGTRLEIK

SEQ ID NO: 67 - protein, 10 aa, Artificial Sequence
FGQGTKVDIK

SEQ ID NO: 68 - protein, 107 aa, Artificial Sequence
EIVLTQSPSSLSASVGDRVTITCLASQTIGTWLAWYQQKPGKSPQLLIYAASTLQSGVPSRFSGSGSGTDFTLTISSLQPEDVATYYCQQYYSTPRTFGQGTKVEIK

SEQ ID NO: 69 - protein, 107 aa, Artificial Sequence
EIVLTQSPSSVSASVGDKLTMTCQASQDIGKHLNWYQQKPGKPPKLLIYGASNLKTGVPSRFSGTGSGTDFTLTISSLQPEDFATYYCQQSYTTPYTFGQGTRLEIK

SEQ ID NO: 70 - protein, 107 aa, Artificial Sequence
EIVLTQSPSSVSASVGDRITITCRASQGIGSWLAWYQQKPGKAPSLLIYAASSLQSGVPSRFSGSGSGTDFTLTISSLQTEDVAVYYCQQYFSTPYTFGQGTKVDIK

SEQ ID NO: 71 - protein, 107 aa, Artificial Sequence
DIQMTQSPSSFSASTGDRVTITCRASQGISSYLAWYQQKPGKAPKLLIYAASRLQSGVPSRFSGSGSGTDFTLTISSLQAEDVAVYYCQQYYSTPYTFGQGTKVDIK

SEQ ID NO: 72 - protein, 107 aa, Artificial Sequence
DIQMTQSPSSLSASVGDRVTIPCRASQGIGKFLAWYQQKPGKAPSLLIYAASSLQSGVPSRFSGSGSGTDFTLTISSLQTEDVAVYYCQQYFSTPYTFGQGTKVDIK

SEQ ID NO: 73 - protein, 107 aa, Artificial Sequence
DIQMTQSPSSLSASVGDRVTITCLASQTIGTWLAWYQQKPGKSPQLLIYAASSLQSGVPSRFSGSGSGTDFTLTISSLQPEDVATYYCQQYYSTPYTFGQGTKVDIK

SEQ ID NO: 74 - protein, 330 aa, Artificial Sequence [sequence omitted]

SEQ ID NO: 75 - protein, 330 aa, Artificial Sequence
ASTKGPSVFPLAPSSKSTSGGTAALGCLVKDYFPEPVTVSWNSGALTSGVHTFPAVLQSSGLYSLSSVVTVPSSSLGTQTYICNVNHKPSNTKVDKKVEPKSCDKTHTCPPCPAPELLGGPSVFLFPPKPKDTLMISRTPEVTCVVVDVSHEDPEVKFNWYVDGVEVHNAKTKPREEQYASTYRVVSVLTVLHQDWLNGKEYKCKVSNKALPAPIEKTISKAKGQPREPQVYTLPPSREEMTKNQVSLTCLVKGFYPSDIAVEWESNGQPENNYKTTPPVLDSDGSFFLYSKLTVDKSRWQQGNVFSCSVMHEALHNHYTQKSLSLSPGK

SEQ ID NO: 76 - protein, 107 aa, Artificial Sequence [sequence omitted]

SEQ ID NO: 77 - protein, 448 aa, Artificial Sequence
EVQLVESGGGLVQPGGSLRLSCAASGFTFSDSWIHWVRQAPGKGLEWVGWISPYGGSTYYADSVKGRFTISADTSKNTAYLQMNSLRAEDTAVYYCARRHWPGGFDYWGQGTLVTVSSASTKGPSVFPLAPSSKSTSGGTAALGCLVKDYFPEPVTVSWNSGALTSGVHTFPAVLQSSGLYSLSSVVTVPSSSLGTQTYICNVNHKPSNTKVDKKVEPKSCDKTHTCPPCPAPELLGGPSVFLFPPKPKDTLMISRTPEVTCVVVDVSHEDPEVKFNWYVDGVEVHNAKTKPREEQYNSTYRVVSVLTVLHQDWLNGKEYKCKVSNKALPAPIEKTISKAKGQPREPQVYTLPPSRDELTKNQVSLTCLVKGFYPSDIAVEWESNGQPENNYKTTPPVLDSDGSFFLYSKLTVDKSRWQQGNVFSCSVMHEALHNHYTQKSLSLSPGK

SEQ ID NO: 78 - protein, 448 aa, Artificial Sequence
EVQLVESGGGLVQPGGSLRLSCAASGFTFSDSWIHWVRQAPGKGLEWVGWISPYGGSTYYADDFRHRFTISADTSKNTAYLQMNSLRAEDTAVYYCARRHWPGGFDYWGQGTLVTVSSASTKGPSVFPLAPSSKSTSGGTAALGCLVKDYFPEPVTVSWNSGALTSGVHTFPAVLQSSGLYSLSSVVTVPSSSLGTQTYICNVNHKPSNTKVDKKVEPKSCDKTHTCPPCPAPELLGGPSVFLFPPKPKDTLMISRTPEVTCVVVDVSHEDPEVKFNWYVDGVEVHNAKTKPREEQYNSTYRVVSVLTVLHQDWLNGKEYKCKVSNKALPAPIEKTISKAKGQPREPQVYTLPPSRDELTKNQVSLTCLVKGFYPSDIAVEWESNGQPENNYKTTPPVLDSDGSFFLYSKLTVDKSRWQQGNVFSCSVMHEALHNHYTQKSLSLSPGK

SEQ ID NO: 79 - protein, 448 aa, Artificial Sequence
EVQLVESGGGLVQPGGSLRLSCAASGFTFSDSWIHWVRQAPGKGLEWVGWISPYGGSTYYADSLGDRFTISADTSKNTAYLQMNSLRAEDTAVYYCARRHWPGGFDYWGQGTLVTVSSASTKGPSVFPLAPSSKSTSGGTAALGCLVKDYFPEPVTVSWNSGALTSGVHTFPAVLQSSGLYSLSSVVTVPSSSLGTQTYICNVNHKPSNTKVDKKVEPKSCDKTHTCPPCPAPELLGGPSVFLFPPKPKDTLMISRTPEVTCVVVDVSHEDPEVKFNWYVDGVEVHNAKTKPREEQYNSTYRVVSVLTVLHQDWLNGKEYKCKVSNKALPAPIEKTISKAKGQPREPQVYTLPPSRDELTKNQVSLTCLVKGFYPSDIAVEWESNGQPENNYKTTPPVLDSDGSFFLYSKLTVDKSRWQQGNVFSCSVMHEALHNHYTQKSLSLSPGK

SEQ ID NO: 80 - protein, 448 aa, Artificial Sequence
EVQLVESGGGLVQPGGSLRLSCAASGFTFSDSWIHWVRQAPGKGLEWVGWISPYGGSTYYADHLSQRFTISADTSKNTAYLQMNSLRAEDTAVYYCARRHWPGGFDYWGQGTLVTVSSASTKGPSVFPLAPSSKSTSGGTAALGCLVKDYFPEPVTVSWNSGALTSGVHTFPAVLQSSGLYSLSSVVTVPSSSLGTQTYICNVNHKPSNTKVDKKVEPKSCDKTHTCPPCPAPELLGGPSVFLFPPKPKDTLMISRTPEVTCVVVDVSHEDPEVKFNWYVDGVEVHNAKTKPREEQYNSTYRVVSVLTVLHQDWLNGKEYKCKVSNKALPAPIEKTISKAKGQPREPQVYTLPPSRDELTKNQVSLTCLVKGFYPSDIAVEWESNGQPENNYKTTPPVLDSDGSFFLYSKLTVDKSRWQQGNVFSCSVMHEALHNHYTQKSLSLSPGK

SEQ ID NO: 81 - protein, 448 aa, Artificial Sequence
EVQLVESGGGLVQPGGSLRLSCAASGFTFSDSWIHWVRQAPGKGLEWVGWISPYGGSTYYADGMRSRFTISADTSKNTAYLQMNSLRAEDTAVYYCARRHWPGGFDYWGQGTLVTVSSASTKGPSVFPLAPSSKSTSGGTAALGCLVKDYFPEPVTVSWNSGALTSGVHTFPAVLQSSGLYSLSSVVTVPSSSLGTQTYICNVNHKPSNTKVDKKVEPKSCDKTHTCPPCPAPELLGGPSVFLFPPKPKDTLMISRTPEVTCVVVDVSHEDPEVKFNWYVDGVEVHNAKTKPREEQYNSTYRVVSVLTVLHQDWLNGKEYKCKVSNKALPAPIEKTISKAKGQPREPQVYTLPPSRDELTKNQVSLTCLVKGFYPSDIAVEWESNGQPENNYKTTPPVLDSDGSFFLYSKLTVDKSRWQQGNVFSCSVMHEALHNHYTQKSLSLSPGK

SEQ ID NO: 82 - protein, 448 aa, Artificial Sequence
EVQLVESGGGLVQPGGSLRLSCAASGFTFSDSWIHWVRQAPGKGLEWVGWISPYGGSTYYADSYRSRFTISADTSKNTAYLQMNSLRAEDTAVYYCARRHWPGGFDYWGQGTLVTVSSASTKGPSVFPLAPSSKSTSGGTAALGCLVKDYFPEPVTVSWNSGALTSGVHTFPAVLQSSGLYSLSSVVTVPSSSLGTQTYICNVNHKPSNTKVDKKVEPKSCDKTHTCPPCPAPELLGGPSVFLFPPKPKDTLMISRTPEVTCVVVDVSHEDPEVKFNWYVDGVEVHNAKTKPREEQYNSTYRVVSVLTVLHQDWLNGKEYKCKVSNKALPAPIEKTISKAKGQPREPQVYTLPPSRDELTKNQVSLTCLVKGFYPSDIAVEWESNGQPENNYKTTPPVLDSDGSFFLYSKLTVDKSRWQQGNVFSCSVMHEALHNHYTQKSLSLSPGK

SEQ ID NO: 83 - protein, 448 aa, Artificial Sequence
EVQLVESGGGLVQPGGSLRLSCAASGFTFSDSWIHWVRQAPGKGLEWVGWISPYGGSTYYADPYVGRFTISADTSKNTAYLQMNSLRAEDTAVYYCARRHWPGGFDYWGQGTLVTVSSASTKGPSVFPLAPSSKSTSGGTAALGCLVKDYFPEPVTVSWNSGALTSGVHTFPAVLQSSGLYSLSSVVTVPSSSLGTQTYICNVNHKPSNTKVDKKVEPKSCDKTHTCPPCPAPELLGGPSVFLFPPKPKDTLMISRTPEVTCVVVDVSHEDPEVKFNWYVDGVEVHNAKTKPREEQYNSTYRVVSVLTVLHQDWLNGKEYKCKVSNKALPAPIEKTISKAKGQPREPQVYTLPPSRDELTKNQVSLTCLVKGFYPSDIAVEWESNGQPENNYKTTPPVLDSDGSFFLYSKLTVDKSRWQQGNVFSCSVMHEALHNHYTQKSLSLSPGK

SEQ ID NO: 84 - protein, 448 aa, Artificial Sequence
EVQLVESGGGLVQPGGSLRLSCAASGFTFSDSWIHWVRQAPGKGLEWVGWISPYGGSTYYADSLKGRFTISADTSKNTAYLQMNSLRAEDTAVYYCARRHWPGGFDYWGQGTLVTVSSASTKGPSVFPLAPSSKSTSGGTAALGCLVKDYFPEPVTVSWNSGALTSGVHTFPAVLQSSGLYSLSSVVTVPSSSLGTQTYICNVNHKPSNTKVDKKVEPKSCDKTHTCPPCPAPELLGGPSVFLFPPKPKDTLMISRTPEVTCVVVDVSHEDPEVKFNWYVDGVEVHNAKTKPREEQYNSTYRVVSVLTVLHQDWLNGKEYKCKVSNKALPAPIEKTISKAKGQPREPQVYTLPPSRDELTKNQVSLTCLVKGFYPSDIAVEWESNGQPENNYKTTPPVLDSDGSFFLYSKLTVDKSRWQQGNVFSCSVMHEALHNHYTQKSLSLSPGK

SEQ ID NO: 85 - protein, 448 aa, Artificial Sequence
EVQLVESGGGLVQPGGSLRLSCAASGFTFSDSWIHWVRQAPGKGLEWVGWISPYGGSTYYADSYRARFTISADTSKNTAYLQMNSLRAEDTAVYYCARRHWPGGFDYWGQGTLVTVSSASTKGPSVFPLAPSSKSTSGGTAALGCLVKDYFPEPVTVSWNSGALTSGVHTFPAVLQSSGLYSLSSVVTVPSSSLGTQTYICNVNHKPSNTKVDKKVEPKSCDKTHTCPPCPAPELLGGPSVFLFPPKPKDTLMISRTPEVTCVVVDVSHEDPEVKFNWYVDGVEVHNAKTKPREEQYNSTYRVVSVLTVLHQDWLNGKEYKCKVSNKALPAPIEKTISKAKGQPREPQVYTLPPSRDELTKNQVSLTCLVKGFYPSDIAVEWESNGQPENNYKTTPPVLDSDGSFFLYSKLTVDKSRWQQGNVFSCSVMHEALHNHYTQKSLSLSPGK

SEQ ID NO: 86 - protein, 448 aa, Artificial Sequence
EVQLVESGGGLVQPGGSLRLSCAASGFTFSDSWIHWVRQAPGKGLEWVGWISPYGGSTYYADYLHGRFTISADTSKNTAYLQMNSLRAEDTAVYYCARRHWPGGFDYWGQGTLVTVSSASTKGPSVFPLAPSSKSTSGGTAALGCLVKDYFPEPVTVSWNSGALTSGVHTFPAVLQSSGLYSLSSVVTVPSSSLGTQTYICNVNHKPSNTKVDKKVEPKSCDKTHTCPPCPAPELLGGPSVFLFPPKPKDTLMISRTPEVTCVVVDVSHEDPEVKFNWYVDGVEVHNAKTKPREEQYNSTYRVVSVLTVLHQDWLNGKEYKCKVSNKALPAPIEKTISKAKGQPREPQVYTLPPSRDELTKNQVSLTCLVKGFYPSDIAVEWESNGQPENNYKTTPPVLDSDGSFFLYSKLTVDKSRWQQGNVFSCSVMHEALHNHYTQKSLSLSPGK

SEQ ID NO: 87 - protein, 448 aa, Artificial Sequence
EVQLVESGGGLVQPGGSLRLSCAASSFSLKDSWIHWVRQAPGKGLEWVGWISPYGGSTYYADSVKGRFTISADTSKNTAYLQMNSLRAEDTAVYYCARRHWPGGFDYWGQGTLVTVSSASTKGPSVFPLAPSSKSTSGGTAALGCLVKDYFPEPVTVSWNSGALTSGVHTFPAVLQSSGLYSLSSVVTVPSSSLGTQTYICNVNHKPSNTKVDKKVEPKSCDKTHTCPPCPAPELLGGPSVFLFPPKPKDTLMISRTPEVTCVVVDVSHEDPEVKFNWYVDGVEVHNAKTKPREEQYNSTYRVVSVLTVLHQDWLNGKEYKCKVSNKALPAPIEKTISKAKGQPREPQVYTLPPSRDELTKNQVSLTCLVKGFYPSDIAVEWESNGQPENNYKTTPPVLDSDGSFFLYSKLTVDKSRWQQGNVFSCSVMHEALHNHYTQKSLSLSPGK

SEQ ID NO: 88 - protein, 448 aa, Artificial Sequence
EVQLVESGGGLVQPGGSLRLSCAASGWATRDSWIHWVRQAPGKGLEWVGWISPYGGSTYYADSVKGRFTISADTSKNTAYLQMNSLRAEDTAVYYCARRHWPGGFDYWGQGTLVTVSSASTKGPSVFPLAPSSKSTSGGTAALGCLVKDYFPEPVTVSWNSGALTSGVHTFPAVLQSSGLYSLSSVVTVPSSSLGTQTYICNVNHKPSNTKVDKKVEPKSCDKTHTCPPCPAPELLGGPSVFLFPPKPKDTLMISRTPEVTCVVVDVSHEDPEVKFNWYVDGVEVHNAKTKPREEQYNSTYRVVSVLTVLHQDWLNGKEYKCKVSNKALPAPIEKTISKAKGQPREPQVYTLPPSRDELTKNQVSLTCLVKGFYPSDIAVEWESNGQPENNYKTTPPVLDSDGSFFLYSKLTVDKSRWQQGNVFSCSVMHEALHNHYTQKSLSLSPGK

SEQ ID NO: 89 - protein, 448 aa, Artificial Sequence
EVQLVESGGGLVQPGGSLRLSCAASGFTFSDSWIHWVRQAPGKGLEWVGWISPYGGSTYYADSVKGRFTISADTSKNTAYLQMNSLRAEDTAVYYCARRHWPGGLLPWGQGTLVTVSSASTKGPSVFPLAPSSKSTSGGTAALGCLVKDYFPEPVTVSWNSGALTSGVHTFPAVLQSSGLYSLSSVVTVPSSSLGTQTYICNVNHKPSNTKVDKKVEPKSCDKTHTCPPCPAPELLGGPSVFLFPPKPKDTLMISRTPEVTCVVVDVSHEDPEVKFNWYVDGVEVHNAKTKPREEQYNSTYRVVSVLTVLHQDWLNGKEYKCKVSNKALPAPIEKTISKAKGQPREPQVYTLPPSRDELTKNQVSLTCLVKGFYPSDIAVEWESNGQPENNYKTTPPVLDSDGSFFLYSKLTVDKSRWQQGNVFSCSVMHEALHNHYTQKSLSLSPGK

SEQ ID NO: 90 - protein, 448 aa, Artificial Sequence
EVQLVESGGGLVQPGGSLRLSCAASGLRPADSWIHWVRQAPGKGLEWVGWISPYGGSTYYADSVKGRFTISADTSKNTAYLQMNSLRAEDTAVYYCARRHWPGGFDYWGQGTLVTVSSASTKGPSVFPLAPSSKSTSGGTAALGCLVKDYFPEPVTVSWNSGALTSGVHTFPAVLQSSGLYSLSSVVTVPSSSLGTQTYICNVNHKPSNTKVDKKVEPKSCDKTHTCPPCPAPELLGGPSVFLFPPKPKDTLMISRTPEVTCVVVDVSHEDPEVKFNWYVDGVEVHNAKTKPREEQYNSTYRVVSVLTVLHQDWLNGKEYKCKVSNKALPAPIEKTISKAKGQPREPQVYTLPPSRDELTKNQVSLTCLVKGFYPSDIAVEWESNGQPENNYKTTPPVLDSDGSFFLYSKLTVDKSRWQQGNVFSCSVMHEALHNHYTQKSLSLSPGK

SEQ ID NO: 91 - protein, 448 aa, Artificial Sequence
EVQLVESGGGLVQPGGSLRLSCAASNSHLRDSWIHWVRQAPGKGLEWVGWISPYGGSTYYADSVKGRFTISADTSKNTAYLQMNSLRAEDTAVYYCARRHWPGGFDYWGQGTLVTVSSASTKGPSVFPLAPSSKSTSGGTAALGCLVKDYFPEPVTVSWNSGALTSGVHTFPAVLQSSGLYSLSSVVTVPSSSLGTQTYICNVNHKPSNTKVDKKVEPKSCDKTHTCPPCPAPELLGGPSVFLFPPKPKDTLMISRTPEVTCVVVDVSHEDPEVKFNWYVDGVEVHNAKTKPREEQYNSTYRVVSVLTVLHQDWLNGKEYKCKVSNKALPAPIEKTISKAKGQPREPQVYTLPPSRDELTKNQVSLTCLVKGFYPSDIAVEWESNGQPENNYKTTPPVLDSDGSFFLYSKLTVDKSRWQQGNVFSCSVMHEALHNHYTQKSLSLSPGK

SEQ ID NO: 92 - protein, 214 aa, Artificial Sequence
EIVLTQSPSSLSASVGDRVTITCLASQTIGTWLAWYQQKPGKSPQLLIYAASTLQSGVPSRFSGSGSGTDFTLTISSLQPEDVATYYCQQYYSTPRTFGQGTKVEIKRTVAAPSVFIFPPSDEQLKSGTASVVCLLNNFYPREAKVQWKVDNALQSGNSQESVTEQDSKDSTYSLSSTLTLSKADYEKHKVYACEVTHQGLSSPVTKSFNRGEC

SEQ ID NO: 93 - protein, 214 aa, Artificial Sequence
EIVLTQSPSSVSASVGDKLTMTCQASQDIGKHLNWYQQKPGKPPKLLIYGASNLKTGVPSRFSGTGSGTDFTLTISSLQPEDFATYYCQQSYTTPYTFGQGTRLEIKRTVAAPSVFIFPPSDEQLKSGTASVVCLLNNFYPREAKVQWKVDNALQSGNSQESVTEQDSKDSTYSLSSTLTLSKADYEKHKVYACEVTHQGLSSPVTKSFNRGEC

SEQ ID NO: 94 - protein, 214 aa, Artificial Sequence
EIVLTQSPSSVSASVGDRITITCRASQGIGSWLAWYQQKPGKAPSLLIYAASSLQSGVPSRFSGSGSGTDFTLTISSLQTEDVAVYYCQQYFSTPYTFGQGTKVDIKRTVAAPSVFIFPPSDEQLKSGTASVVCLLNNFYPREAKVQWKVDNALQSGNSQESVTEQDSKDSTYSLSSTLTLSKADYEKHKVYACEVTHQGLSSPVTKSFNRGEC

SEQ ID NO: 95 - protein, 214 aa, Artificial Sequence
DIQMTQSPSSFSASTGDRVTITCRASQGISSYLAWYQQKPGKAPKLLIYAASRLQSGVPSRFSGSGSGTDFTLTISSLQAEDVAVYYCQQYYSTPYTFGQGTKVDIKRTVAAPSVFIFPPSDEQLKSGTASVVCLLNNFYPREAKVQWKVDNALQSGNSQESVTEQDSKDSTYSLSSTLTLSKADYEKHKVYACEVTHQGLSSPVTKSFNRGEC

SEQ ID NO: 96 - protein, 214 aa, Artificial Sequence
DIQMTQSPSSLSASVGDRVTIPCRASQGIGKFLAWYQQKPGKAPSLLIYAASSLQSGVPSRFSGSGSGTDFTLTISSLQTEDVAVYYCQQYFSTPYTFGQGTKVDIKRTVAAPSVFIFPPSDEQLKSGTASVVCLLNNFYPREAKVQWKVDNALQSGNSQESVTEQDSKDSTYSLSSTLTLSKADYEKHKVYACEVTHQGLSSPVTKSFNRGEC

SEQ ID NO: 97 - protein, 214 aa, Artificial Sequence
DIQMTQSPSSLSASVGDRVTITCLASQTIGTWLAWYQQKPGKSPQLLIYAASSLQSGVPSRFSGSGSGTDFTLTISSLQPEDVATYYCQQYYSTPYTFGQGTKVDIKRTVAAPSVFIFPPSDEQLKSGTASVVCLLNNFYPREAKVQWKVDNALQSGNSQESVTEQDSKDSTYSLSSTLTLSKADYEKHKVYACEVTHQGLSSPVTKSFNRGEC

SEQ ID NO: 98 - protein, 238 aa, Artificial Sequence
MRIFAVFIFMTYWHLLNAFTVTVPKDLYVVEYGSNMTIECKFPVEKQLDLAALIVYWEMEDKNIIQFVHGEEDLKVQHSSYRQRARLLKDQLSLGNAALQITDVKLQDAGVYRCMISYGGADYKRITVKVNAPYNKINQRILVVDPVTSEHELTCQAEGYPKAEVIWTSSDHQVLSGKTTTTNSKREEKLFNVTSTLRINTTTNEIFYCTFRRLDPEENHTAELVIPELPLAHPPNER

SEQ ID NO: 99 - DNA, 1344 bp, Artificial Sequence
gaggtgcagctggtggaatccggcggagggctggtgcagccaggtggctctctgagactgagttgcgccgcttcaggattcaccttttccgactcttggattcactgggtgcgccaggcccccggaaagggactggagtgggtcggttggatttctccttacggagggagtacatactatgccgacagtcttggtgatcgattcactatctccgctgatactagcaaaaacaccgcatatctgcagatgaactccctgagggcagaagacacagccgtctactattgtgcaaggcggcattggcccggtggctttgattactggggtcagggtaccctggttaccgttagcagcgcgagcaccaaaggcccgagcgtgtttccgctggccccgagcagcaaaagcaccagcggtggcaccgcagcgctgggttgcctggtgaaagattatttcccggaaccggtgacggtgtcgtggaactcaggcgccctgaccagcggcgtgcacaccttcccggctgtcctacagtcctcaggactctactccctcagcagcgtggtgaccgtgccctccagcagcttgggcacccagacctacatctgcaacgtgaatcacaagcccagcaacaccaaggtggacaagaaagttgagcccaaatcttgtgacaaaactcacacatgcccaccgtgcccagcacctgaactcctggggggaccgtcagtcttcctcttccccccaaaacccaaggacaccctcatgatctcccggacccctgaggtcacatgcgtggtggtggacgtgagccacgaagaccctgaggtcaagttcaactggtacgtggacggcgtggaggtgcataatgccaagacaaagccgcgggaggagcagtacaacagcacgtaccgggtggtcagcgtcctcaccgtcctgcaccaggactggctgaatggcaaggagtacaagtgcaaggtctccaacaaagccctcccagcccccatcgagaaaaccatctccaaagccaaagggcagccccgagaaccacaggtgtacaccctgcccccatcccgggatgagctgaccaagaaccaggtcagcctgacctgcctggtcaaaggcttctatcccagcgacatcgccgtggagtgggagagcaatgggcagccggagaacaactacaagaccacgcctcccgtgctggactccgacggctccttcttcctctacagcaagctcaccgtggacaagagcaggtggcagcaggggaacgtcttctcatgctccgtgatgcatgaggctctgcacaaccactacacgcagaagagcctctccctgtctccgggtaaa

SEQ ID NO: 100 - DNA, 1344 bp, Artificial Sequence
gaggtgcagctggtggaatccggcggagggctggtgcagccaggtggctctctgagactgagttgcgccgcttcaggattcaccttttccgactcttggattcactgggtgcgccaggcccccggaaagggactggagtgggtcggttggatttctccttacggagggagtacatactatgccgactcttataggtcgcgattcactatctccgctgatactagcaaaaacaccgcatatctgcagatgaactccctgagggcagaagacacagccgtctactattgtgcaaggcggcattggcccggtggctttgattactggggtcagggtaccctggttaccgttagcagcgcgagcaccaaaggcccgagcgtgtttccgctggccccgagcagcaaaagcaccagcggtggcaccgcagcgctgggttgcctggtgaaagattatttcccggaaccggtgacggtgtcgtggaactcaggcgccctgaccagcggcgtgcacaccttcccggctgtcctacagtcctcaggactctactccctcagcagcgtggtgaccgtgccctccagcagcttgggcacccagacctacatctgcaacgtgaatcacaagcccagcaacaccaaggtggacaagaaagttgagcccaaatcttgtgacaaaactcacacatgcccaccgtgcccagcacctgaactcctggggggaccgtcagtcttcctcttccccccaaaacccaaggacaccctcatgatctcccggacccctgaggtcacatgcgtggtggtggacgtgagccacgaagaccctgaggtcaagttcaactggtacgtggacggcgtggaggtgcataatgccaagacaaagccgcgggaggagcagtacaacagcacgtaccgggtggtcagcgtcctcaccgtcctgcaccaggactggctgaatggcaaggagtacaagtgcaaggtctccaacaaagccctcccagcccccatcgagaaaaccatctccaaagccaaagggcagccccgagaaccacaggtgtacaccctgcccccatcccgggatgagctgaccaagaaccaggtcagcctgacctgcctggtcaaaggcttctatcccagcgacatcgccgtggagtgggagagcaatgggcagccggagaacaactacaagaccacgcctcccgtgctggactccgacggctccttcttcctctacagcaagctcaccgtggacaagagcaggtggcagcaggggaacgtcttctcatgctccgtgatgcatgaggctctgcacaaccactacacgcagaagagcctctccctgtctccgggtaaa

SEQ ID NO: 101 - DNA, 642 bp, Artificial Sequence
gaaattgtgctgactcagtctccatcctccctgtctgcatctgtaggagacagagtcaccatcacttgcctggcaagtcagaccattggtacatggttagcatggtatcagcagaaaccagggaaatctcctcagctcctgatctatgctgcatccactttgcaatcaggggtcccatctcggttcagtggcagtggatctgggacagatttcactctcaccatcagcagcctgcagcctgaagatgttgcaacttattactgtcagcaatattatagtactcctcggacgttcggccaagggaccaaggtggagattaaacgtacggtggctgcaccatctgtcttcatcttcccgccatctgatgagcagttgaaatctggaactgcctctgttgtgtgcctgctgaataacttctatcccagagaggccaaagtacagtggaaggtggataacgccctccaatcgggtaactcccaggagagtgtcacagagcaggacagcaaggacagcacctacagcctcagcagcaccctgacgctgagcaaagcagactacgagaaacacaaagtctacgcctgcgaagtcacccatcagggcctgagctcgcccgtcacaaagagcttcaacaggggagagtgt

SEQ ID NO: 102 - DNA, 57 bp, Artificial Sequence
atggagtttgggctgagctgggttttccttgttgctatattaaaaggtgtccagtgt

SEQ ID NO: 103 - DNA, 66 bp, Artificial Sequence
atggacatgagggtgctggcccagctgctgggactcctcctgctgtgcttcccaggcgccagatgc

SEQ ID NO: 104 - protein, 19 aa, Artificial Sequence
MEFGLSWVFLVAILKGVQC

SEQ ID NO: 105 - protein, 22 aa, Artificial Sequence
MDMRVLAQLLGLLLLCFPGARC

SEQ ID NO: 106 - protein, 15 aa, Artificial Sequence
GGGGSGGGGSGGGGS

SEQ ID NO: 107 - DNA, 45 bp, Artificial Sequence
ggtggaggcggttcaggcggaggtggctctggcggtggcggatcg